European Patent Specification EP 3 558 339 B1, published January 24, 2024. Title: T-Cell Modulatory Polypeptides and Methods of Use Thereof. Applicant: Cue Biopharma, Inc. Application EP17884258.9. The sequence listing filed with the application follows.

SEQUENCE LISTING (100 sequences)

SEQ ID NO: 1 - protein, 133 aa, Homo sapiens [sequence omitted]

SEQ ID NO: 2 - protein, 4 aa, Artificial sequence
  Synthetic Polypeptide Sequence
GGSG

SEQ ID NO: 3 - protein, 5 aa, Artificial sequence
  Synthetic Polypeptide Sequence
GGSGG

SEQ ID NO: 4 - protein, 5 aa, Artificial sequence
  Synthetic Polypeptide Sequence
GSGSG

SEQ ID NO: 5 - protein, 5 aa, Artificial sequence
  Synthetic Polypeptide Sequence
GSGGG

SEQ ID NO: 6 - protein, 5 aa, Artificial sequence
  Synthetic Polypeptide Sequence
GGGSG

SEQ ID NO: 7 - protein, 5 aa, Artificial sequence
  Synthetic Polypeptide Sequence
GSSSG

SEQ ID NO: 8 - protein, 5 aa, Artificial sequence
  Synthetic Polypeptide Sequence
GSSSS

SEQ ID NO: 9 - protein, 5 aa, Artificial sequence
  Synthetic Polypeptide Sequence
GGGGS

SEQ ID NO: 10 - protein, 15 aa, Artificial sequence
  Synthetic Polypeptide Sequence
GCGASGGGGSGGGGS

SEQ ID NO: 11 - protein, 9 aa, Artificial sequence
  Synthetic Polypeptide Sequence
LLMGTLGIV

SEQ ID NO: 12 - protein, 8 aa, Artificial sequence
  Synthetic Polypeptide Sequence
TLGIVCPI

SEQ ID NO: 13 - protein, 10 aa, Artificial sequence
  Synthetic Polypeptide Sequence
YMLDLQPETT

SEQ ID NO: 14 - protein, 276 aa, Homo sapiens [sequence omitted]

SEQ ID NO: 15 - protein, 274 aa, Mus musculus
GPHSLRYFVTAVSRPGLGEPRFIAVGYVDDTQFVRFDSDADNPRFEPRAPWMEQEGPEYWEEQTQRAKSDEQWFRVSLRTAQRYYNQSKGGSHTFQRMFGCDVGSDWRLLRGYQQFAYDGRDYIALNEDLKTWTAADTAALITRRKWEQAGDAEYYRAYLEGECVEWLRRYLELGNETLLRTDSPKAHVTYHPRSQVDVTLRCWALGFYPADITLTWQLNGEDLTQDMELVETRPAGDGTFQKWAAVVVPLGKEQNYTCHVHHKGLPEPLTLRW

SEQ ID NO: 16 - protein, 99 aa, Artificial sequence [sequence omitted]

SEQ ID NO: 17 - protein, 99 aa, Artificial sequence
  Synthetic Polypeptide Sequence
IQRTPKIQVYSCHPAENGKSNFLNCYVSGFHPSDIEVDLLKNGERIEKVEHSDLSFSKDWSFYLLYYTEFTPTEKDEYACRVNHVTLSQPKIVKWDRDM

SEQ ID NO: 18 - protein, 276 aa, Homo sapiens
GSHSMRYFFTSVSRPGRGEPRFIAVGYVDDTQFVRFDSDAASQRMEPRAPWIEQEGPEYWDGETRKVKAHSQTHRVDLGTLRGYYNQSEAGSHTVQRMYGCDVGSDWRFLRGYHQYAYDGKDYIALKEDLRSWTAADMAAQTTKHKWEAAHVAEQLRAYLEGTCVEWLRRYLENGKETLQRTDAPKTHMTHHAVSDHEATLRCWALSFYPAEITLTWQRDGEDQTQDTELVETRPCGDGTFQKWAAVVVPSGQEQRYTCHVQHEGLPKPLTLRWEP

SEQ ID NO: 19 - protein, 275 aa, Homo sapiens
GSHSMRYFFTSVSRPGRGEPRFIAVGYVDDTQFVRFDSDAASQRMEPRAPWIEQEGPEYWDGETRKVKAHSQTHRVDLGTLRGAYNQSEAGSHTVQRMYGCDVGSDWRFLRGYHQYAYDGKDYIALKEDLRSWTAADMAAQTTKHKWEAAHVAEQLRAYLEGTCVEWLRRYLENGKETLQRTDAPKTHMTHHAVSDHEATLRCWALSFYPAEITLTWQRDGEDQTQDTELVETRPCGDGTFQKWAAVVVPSGQEQRYTCHVQHEGLPKPLTLRWE

SEQ ID NO: 20 - protein, 9 aa, Artificial sequence
  Synthetic Polypeptide Sequence
YPYDVPDYA

SEQ ID NO: 21 - protein, 8 aa, Artificial sequence
  Synthetic Polypeptide Sequence
DYKDDDDK

SEQ ID NO: 22 - protein, 10 aa, Artificial sequence
  Synthetic Polypeptide Sequence
EQKLISEEDL

SEQ ID NO: 23 - protein, 5 aa, Artificial sequence
  Synthetic Polypeptide Sequence
HHHHH

SEQ ID NO: 24 - protein, 6 aa, Artificial sequence
  Synthetic Polypeptide Sequence
HHHHHH

SEQ ID NO: 25 - protein, 8 aa, Artificial sequence
  Synthetic Polypeptide Sequence
WSHPQFEK

SEQ ID NO: 26 - protein, 5 aa, Artificial sequence
  Synthetic Polypeptide Sequence
RYIRS

SEQ ID NO: 27 - protein, 17 aa, Artificial sequence
  Synthetic Polypeptide Sequence
WEAAAREACCRECCARA

SEQ ID NO: 28 - protein, 5 aa, Artificial sequence
  Synthetic Polypeptide Sequence
AAAGG

SEQ ID NO: 29 - protein, 8 aa, Artificial sequence
  Synthetic Polypeptide Sequence
LEVLFQGP

SEQ ID NO: 30 - protein, 7 aa, Artificial sequence
  Synthetic Polypeptide Sequence
ENLYTQS

SEQ ID NO: 31 - protein, 5 aa, Artificial sequence
  Synthetic Polypeptide Sequence
DDDDK

SEQ ID NO: 32 - protein, 4 aa, Artificial sequence
  Synthetic Polypeptide Sequence
LVPR

SEQ ID NO: 33 - protein, 22 aa, Artificial sequence
  Synthetic Polypeptide Sequence
GSGATNFSLLKQAGDVEENPGP

SEQ ID NO: 34 - protein, 21 aa, Artificial sequence
  Synthetic Polypeptide Sequence
GSGEGRGSLLTCGDVEENPGP

SEQ ID NO: 35 - protein, 23 aa, Artificial sequence
  Synthetic Polypeptide Sequence
GSGQCTNYALLKLAGDVESNPGP

SEQ ID NO: 36 - protein, 25 aa, Artificial sequence
  Synthetic Polypeptide Sequence
GSGVKQTLNFDLLKLAGDVESNPGP

SEQ ID NO: 37 - protein, 9 aa, Artificial sequence
  Synthetic Polypeptide Sequence
NLVPMVATV

SEQ ID NO: 38 - protein, 133 aa, Homo sapiens
  MISC_FEATURE (42)..(42): Xaa is an amino acid other than a phenylalanine
APTSSSTKKTQLQLEHLLLDLQMILNGINNYKNPKLTRMLTXKFYMPKKATELKHLQCLEEELKPLEEVLNLAQSKNFHLRPRDLISNINVIVLELKGSETTFMCEYADETATIVEFLNRWITFCQSIISTLT

SEQ ID NO: 39 - protein, 133 aa, Homo sapiens
  MISC_FEATURE (20)..(20): Xaa is an amino acid other than an aspartic acid
APTSSSTKKTQLQLEHLLLXLQMILNGINNYKNPKLTRMLTFKFYMPKKATELKHLQCLEEELKPLEEVLNLAQSKNFHLRPRDLISNINVIVLELKGSETTFMCEYADETATIVEFLNRWITFCQSIISTLT

SEQ ID NO: 40 - protein, 133 aa, Homo sapiens
  MISC_FEATURE (15)..(15): Xaa is an amino acid other than a glutamic acid
APTSSSTKKTQLQLXHLLLDLQMILNGINNYKNPKLTRMLTFKFYMPKKATELKHLQCLEEELKPLEEVLNLAQSKNFHLRPRDLISNINVIVLELKGSETTFMCEYADETATIVEFLNRWITFCQSIISTLT

SEQ ID NO: 41 - protein, 133 aa, Homo sapiens
  MISC_FEATURE (16)..(16): Xaa is an amino acid other than a histidine
APTSSSTKKTQLQLEXLLLDLQMILNGINNYKNPKLTRMLTFKFYMPKKATELKHLQCLEEELKPLEEVLNLAQSKNFHLRPRDLISNINVIVLELKGSETTFMCEYADETATIVEFLNRWITFCQSIISTLT

SEQ ID NO: 42 - protein, 133 aa, Homo sapiens
  MISC_FEATURE (45)..(45): Xaa is an amino acid other than a tyrosine
APTSSSTKKTQLQLEHLLLDLQMILNGINNYKNPKLTRMLTFKFXMPKKATELKHLQCLEEELKPLEEVLNLAQSKNFHLRPRDLISNINVIVLELKGSETTFMCEYADETATIVEFLNRWITFCQSIISTLT

SEQ ID NO: 43 - protein, 133 aa, Homo sapiens
  MISC_FEATURE (126)..(126): Xaa is an amino acid other than a glutamine
APTSSSTKKTQLQLEHLLLDLQMILNGINNYKNPKLTRMLTFKFYMPKKATELKHLQCLEEELKPLEEVLNLAQSKNFHLRPRDLISNINVIVLELKGSETTFMCEYADETATIVEFLNRWITFCXSIISTLT

SEQ ID NO: 44 - protein, 133 aa, Homo sapiens
  MISC_FEATURE (16)..(16): Xaa is an amino acid other than a histidine
  MISC_FEATURE (42)..(42): Xaa is an amino acid other than a phenylalanine
APTSSSTKKTQLQLEXLLLDLQMILNGINNYKNPKLTRMLTXKFYMPKKATELKHLQCLEEELKPLEEVLNLAQSKNFHLRPRDLISNINVIVLELKGSETTFMCEYADETATIVEFLNRWITFCQSIISTLT

SEQ ID NO: 45 - protein, 133 aa, Homo sapiens
  MISC_FEATURE (20)..(20): Xaa is an amino acid other than an aspartic acid
  MISC_FEATURE (42)..(42): Xaa is an amino acid other than a phenylalanine
APTSSSTKKTQLQLEHLLLXLQMILNGINNYKNPKLTRMLTXKFYMPKKATELKHLQCLEEELKPLEEVLNLAQSKNFHLRPRDLISNINVIVLELKGSETTFMCEYADETATIVEFLNRWITFCQSIISTLT

SEQ ID NO: 46 - protein, 133 aa, Homo sapiens
  MISC_FEATURE (15)..(15): Xaa is an amino acid other than a glutamic acid
  MISC_FEATURE (20)..(20): Xaa is an amino acid other than a aspartic acid
  MISC_FEATURE (42)..(42): Xaa is an amino acid other than a phenylalanine
APTSSSTKKTQLQLXHLLLXLQMILNGINNYKNPKLTRMLTXKFYMPKKATELKHLQCLEEELKPLEEVLNLAQSKNFHLRPRDLISNINVIVLELKGSETTFMCEYADETATIVEFLNRWITFCQSIISTLT

SEQ ID NO: 47 - protein, 133 aa, Homo sapiens
  MISC_FEATURE (16)..(16): Xaa is an amino acid other than a histidine
  MISC_FEATURE (20)..(20): Xaa is an amino acid other than an aspartic acid
  MISC_FEATURE (42)..(42): Xaa is an amino acid other than a phenylalanine
APTSSSTKKTQLQLEXLLLXLQMILNGINNYKNPKLTRMLTXKFYMPKKATELKHLQCLEEELKPLEEVLNLAQSKNFHLRPRDLISNINVIVLELKGSETTFMCEYADETATIVEFLNRWITFCQSIISTLT

SEQ ID NO: 48 - protein, 133 aa, Homo sapiens
  MISC_FEATURE (20)..(20): Xaa is an amino acid other than an aspartic acid
  MISC_FEATURE (42)..(42): Xaa is an amino acid other than a phenylalanine
  MISC_FEATURE (126)..(126): Xaa is an amino acid other than a glutamine
APTSSSTKKTQLQLEHLLLXLQMILNGINNYKNPKLTRMLTXKFYMPKKATELKHLQCLEEELKPLEEVLNLAQSKNFHLRPRDLISNINVIVLELKGSETTFMCEYADETATIVEFLNRWITFCXSIISTLT

SEQ ID NO: 49 - protein, 133 aa, Homo sapiens
  MISC_FEATURE (20)..(20): Xaa is an amino acid other than an aspartic acid
  MISC_FEATURE (42)..(42): Xaa is an amino acid other than a phenylalanine
  MISC_FEATURE (45)..(45): Xaa is an amino acid other than a tyrosine
APTSSSTKKTQLQLEHLLLXLQMILNGINNYKNPKLTRMLTXKFXMPKKATELKHLQCLEEELKPLEEVLNLAQSKNFHLRPRDLISNINVIVLELKGSETTFMCEYADETATIVEFLNRWITFCQSIISTLT

SEQ ID NO: 50 - protein, 133 aa, Homo sapiens
  MISC_FEATURE (16)..(16): Xaa is an amino acid other than a histidine
  MISC_FEATURE (20)..(20): Xaa is an amino acid other than an aspartic acid
  MISC_FEATURE (42)..(42): Xaa is an amino acid other than a phenylalanine
  MISC_FEATURE (45)..(45): Xaa is an amino acid other than a tyrosine
APTSSSTKKTQLQLEXLLLXLQMILNGINNYKNPKLTRMLTXKFXMPKKATELKHLQCLEEELKPLEEVLNLAQSKNFHLRPRDLISNINVIVLELKGSETTFMCEYADETATIVEFLNRWITFCQSIISTLT

SEQ ID NO: 51 - protein, 133 aa, Homo sapiens
  MISC_FEATURE (20)..(20): Xaa is an amino acid other than an aspartic acid
  MISC_FEATURE (42)..(42): Xaa is an amino acid other than a phenylalanine
  MISC_FEATURE (45)..(45): Xaa is an amino acid other than a tyrosine
  MISC_FEATURE (126)..(126): Xaa is an amino acid other than a glutamine
APTSSSTKKTQLQLEHLLLXLQMILNGINNYKNPKLTRMLTXKFXMPKKATELKHLQCLEEELKPLEEVLNLAQSKNFHLRPRDLISNINVIVLELKGSETTFMCEYADETATIVEFLNRWITFCXSIISTLT

SEQ ID NO: 52 - protein, 133 aa, Homo sapiens
  MISC_FEATURE (16)..(16): Xaa is an amino acid other than a histidine
  MISC_FEATURE (20)..(20): Xaa is an amino acid other than an aspartic acid
  MISC_FEATURE (42)..(42): Xaa is an amino acid other than a phenylalanine
  MISC_FEATURE (45)..(45): Xaa is an amino acid other than a tyrosine
  MISC_FEATURE (126)..(126): Xaa is an amino acid other than a glutamine
APTSSSTKKTQLQLEXLLLXLQMILNGINNYKNPKLTRMLTXKFXMPKKATELKHLQCLEEELKPLEEVLNLAQSKNFHLRPRDLISNINVIVLELKGSETTFMCEYADETATIVEFLNRWITFCXSIISTLT

SEQ ID NO: 53 - protein, 133 aa, Homo sapiens
  MISC_FEATURE (16)..(16): Xaa is an amino acid other than a histidine
  MISC_FEATURE (42)..(42): Xaa is an amino acid other than a phenylalanine
  MISC_FEATURE (126)..(126): Xaa is an amino acid other than a glutamine
APTSSSTKKTQLQLEXLLLDLQMILNGINNYKNPKLTRMLTXKFYMPKKATELKHLQCLEEELKPLEEVLNLAQSKNFHLRPRDLISNINVIVLELKGSETTFMCEYADETATIVEFLNRWITFCXSIISTLT

SEQ ID NO: 54 - protein, 272 aa, Homo sapiens
MDSYLLMWGLLTFIMVPGCQAELCDDDPPEIPHATFKAMAYKEGTMLNCECKRGFRRIKSGSLYMLCTGNSSHSSWDNQCQCTSSATRNTTKQVTPQPEEQKERKTTEMQSPMQPVDQASLPGHCREPPPWENEATERIYHFVVGQMVYYQCVQGYRALHRGPAESVCKMTHGKTRWTQPQLICTGEMETSQFPGEEKPQASPEGRPESETSCLVTTTDFQIQTEMAATMETSIFTTEYQVAVAGCVFLLISVLLLSGLTWQRRQRKSRRTI

SEQ ID NO: 55 - protein, 491 aa, Homo sapiens
MAAPALSWRLPLLILLLPLATSWASAAVNGTSQFTCFYNSRANISCVWSQDGALQDTSCQVHAWPDRRRWNQTCELLPVSQASWACNLILGAPDSQKLTTVDIVTLRVLCREGVRWRVMAAPLLTLKQKQEWICLETLTPDTQYEFQVRVKPLQGEFTTWSPWSQPLAFRTKPAALGKDTIPWLGHLLVGLSGAFGFIILVYLLINCRNTGPWLKKVLKCNTPDPSKFFSQLSSEHGGDVQKWLSSPFPSSSFSPGGLAPEISPLEVLERDKVTQLLLQQDKVPEPASLSSNHSLTSCFTNQGYFFFHLPDALEIEACQVYFTYDPYSEEDPDEGVAGAPTGSSPQPLQPLSGEDDAYCTFPSRDDLLLFSPSLLGGPSPPSTAPGGSGAGEERMPPSLQERVPRDWDPQPLGPPTPGVPDLVDFQPPPELVLREAGEEVPDAGPREGVSFPWSRPPGQGEFRALNARLPLNTDAYLSLQELQGQDPTHLV

SEQ ID NO: 56 - protein, 369 aa, Homo sapiens
MLKPSLPFTSLLFLQLPLLGVGLNTTILTPNGNEDTTADFFLTTMPTDSLSVSTLPLPEVQCFVFNVEYMNCTWNSSSEPQPTNLTLHYWYKNSDNDKVQKCSHYLFSEEITSGCQLQKKEIHLYQTFVVQLQDPREPRRQATQMLKLQNLVIPWAPENLTLHKLSESQLELNWNNRFLNHCLEHLVQYRTDWDHSWTEQSVDYRHKFSLPSVDGQKRYTFRVRSRFNPLCGSAQHWSEWSHPIHWGSNTSKENPFLFALEAVVISVGSMGLIISLLCVYFWLERTMPRIPTLKNLEDLVTEYHGNFSAWSGVSKGLAESLQPDYSERLCLVSEIPPKGGALGEGPGASPCNQHSPYWAPPCYTLKPET

SEQ ID NO: 57 - protein, 227 aa, Homo sapiens
DKTHTCPPCPAPELLGGPSVFLFPPKPKDTLMISRTPEVTCVVVDVSHEDPEVKFNWYVDGVEVHNAKTKPREEQYNSTYRVVSVLTVLHQDWLNGKEYKCKVSNKALPAPIEKTISKAKGQPREPQVYTLPPSRDELTKNQVSLTCLVKGFYPSDIAVEWESNGQPENNYKTTPPVLDSDGSFFLYSKLTVDKSRWQQGNVFSCSVMHEALHNHYTQKSLSLSPGK

SEQ ID NO: 58 - protein, 325 aa, Homo sapiens
STKGPSVFPLAPCSRSTSESTAALGCLVKDYFPEPVTVSWNSGALTSGVHTFPAVLQSSGLYSLSSVVTVPSSNFGTQTYTCNVDHKPSNTKVDKTVERKCCVECPPCPAPPVAGPSVFLFPPKPKDTLMISRTPEVTCVVVDVSHEDPEVQFNWYVDGVEVHNAKTKPREEQFNSTFRVVSVLTVVHQDWLNGKEYKCKVSNKGLPAPIEKTISKTKGQPREPQVYTLPPSREEMTKNQVSLTCLVKGFYPSDIAVEWESNGQPENNYKTTPPMLDSDGSFFLYSKLTVDKSRWQQGNVFSCSVMHEALHNHYTQKSLSLSPGK

SEQ ID NO: 59 - protein, 246 aa, Homo sapiens
HKPSNTKVDKRVELKTPLGDTTHTCPPCPAPELLGGPSVFLFPPKPKDTLMISRTPEVTCVVVDVSHEDPEVKFNWYVDGVEVHNAKTKPREEQYNSTYRVVSVLTVLHQDWLNGKEYKCKVSNKALPAPIEKTISKAKGQPREPQVYTLPPSRDELTKNQVSLTCLVKGFYPSDIAVEWESNGQPENNYKTTPPVLDSDGSFFLYSKLTVDKSRWQQGNVFSCSVMHEALHNHYTQKSLSLSPGK

SEQ ID NO: 60 - protein, 383 aa, Homo sapiens
PTKAPDVFPIISGCRHPKDNSPVVLACLITGYHPTSVTVTWYMGTQSQPQRTFPEIQRRDSYYMTSSQLSTPLQQWRQGEYKCVVQHTASKSKKEIFRWPESPKAQASSVPTAQPQAEGSLAKATTAPATTRNTGRGGEEKKKEKEKEEQEERETKTPECPSHTQPLGVYLLTPAVQDLWLRDKATFTCFVVGSDLKDAHLTWEVAGKVPTGGVEEGLLERHSNGSQSQHSRLTLPRSLWNAGTSVTCTLNHPSLPPQRLMALREPAAQAPVKLSLNLLASSDPPEAASWLLCEVSGFSPPNILLMWLEDQREVNTSGFAPARPPPQPRSTTFWAWSVLRVPAPPSPQPATYTCVVSHEDSRTLLNASRSLEVSYVTDHGPMK

SEQ ID NO: 61 - protein, 276 aa, Homo sapiens
VTSTLTIKZSDWLGESMFTCRVDHRGLTFQQNASSMCVPDQDTAIRVFAIPPSFASIFLTKSTKLTCLVTDLTTYBSVTISWTREENGAVKTHTNISESHPNATFSAVGEASICEDBDWSGERFTCTVTHTDLPSPLKQTISRPKGVALHRPBVYLLPPARZZLNLRESATITCLVTGFSPADVFVEWMQRGEPLSPQKYVTSAPMPEPQAPGRYFAHSILTVSEEEWNTGGTYTCVVAHEALPNRVTERTVDKSTGKPTLYNVSLVMSDTAGTCY

SEQ ID NO: 62 - protein, 353 aa, Homo sapiens
ASPTSPKVFPLSLCSTQPDGNVVIACLVQGFFPQEPLSVTWSESGQGVTARNFPPSQDASGDLYTTSSQLTLPATQCLAGKSVTCHVKHYTNPSQDVTVPCPVPSTPPTPSPSTPPTPSPSCCHPRLSLHRPALEDLLLGSEANLTCTLTGLRDASGVTFTWTPSSGKSAVQGPPERDLCGCYSVSSVLPGCAEPWNHGKTFTCTAAYPESKTPLTATLSKSGNTFRPEVHLLPPPSEELALNELVTLTCLARGFSPKDVLVRWLQGSQELPREKYLTWASRQEPSQGTTTFAVTSILRVAAEDWKKGDTFSCMVGHEALPLAFTQKTIDRLAGKPTHVNVSVVMAEVDGTCY

SEQ ID NO: 63 - protein, 222 aa, Homo sapiens
ADPCDSNPRGVSAYLSRPSPFDLFIRKSPTITCLVVDLAPSKGTVNLTWSRASGKPVNHSTRKEEKQRNGTLTVTSTLPVGTRDWIEGETYQCRVTHPHLPRALMRSTTKTSGPRAAPEVYAFATPEWPGSRDKRTLACLIQNFMPEDISVQWLHNEVQLPDARHSTTQPRKTKGSGFFVFSRLEVTRAEWEQKDEFICRAVHEAASPSQTVQRAVSVNPGK

SEQ ID NO: 64 - protein, 327 aa, Homo sapiens
ASTKGPSVFPLAPCSRSTSESTAALGCLVKDYFPEPVTVSWNSGALTSGVHTFPAVLQSSGLYSLSSVVTVPSSSLGTKTYTCNVDHKPSNTKVDKRVESKYGPPCPSCPAPEFLGGPSVFLFPPKPKDTLMISRTPEVTCVVVDVSQEDPEVQFNWYVDGVEVHNAKTKPREEQFNSTYRVVSVLTVLHQDWLNGKEYKCKVSNKGLPSSIEKTISKAKGQPREPQVYTLPPSQEEMTKNQVSLTCLVKGFYPSDIAVEWESNGQPENNYKTTPPVLDSDGSFFLYSRLTVDKSRWQEGNVFSCSVMHEALHNHYTQKSLSLSLGK

SEQ ID NO: 65 - protein, 365 aa, Homo sapiens
MAVMAPRTLLLLLSGALALTQTWAGSHSMRYFFTSVSRPGRGEPRFIAVGYVDDTQFVRFDSDAASQKMEPRAPWIEQEGPEYWDQETRNMKAHSQTDRANLGTLRGYYNQSEDGSHTIQIMYGCDVGPDGRFLRGYRQDAYDGKDYIALNEDLRSWTAADMAAQITKRKWEAVHAAEQRRVYLEGRCVDGLRRYLENGKETLQRTDPPKTHMTHHPISDHEATLRCWALGFYPAEITLTWQRDGEDQTQDTELVETRPAGDGTFQKWAAVVVPSGEEQRYTCHVQHEGLPKPLTLRWELSSQPTIPIVGIIAGLVLLGAVITGAVVAAVMWRRKSSDRKGGSYTQAASSDSAQGSDVSLTACKV

SEQ ID NO: 66 - protein, 362 aa, Homo sapiens
MLVMAPRTVLLLLSAALALTETWAGSHSMRYFYTSVSRPGRGEPRFISVGYVDDTQFVRFDSDAASPREEPRAPWIEQEGPEYWDRNTQIYKAQAQTDRESLRNLRGYYNQSEAGSHTLQSMYGCDVGPDGRLLRGHDQYAYDGKDYIALNEDLRSWTAADTAAQITQRKWEAAREAEQRRAYLEGECVEWLRRYLENGKDKLERADPPKTHVTHHPISDHEATLRCWALGFYPAEITLTWQRDGEDQTQDTELVETRPAGDRTFQKWAAVVVPSGEEQRYTCHVQHEGLPKPLTLRWEPSSQSTVPIVGIVAGLAVLAVVVIGAVVAAVMCRRKSSGGKGGSYSQAACSDSAQGSDVSLTA

SEQ ID NO: 67 - protein, 366 aa, Homo sapiens
MRVMAPRALLLLLSGGLALTETWACSHSMRYFDTAVSRPGRGEPRFISVGYVDDTQFVRFDSDAASPRGEPRAPWVEQEGPEYWDRETQNYKRQAQADRVSLRNLRGYYNQSEDGSHTLQRMYGCDLGPDGRLLRGYDQSAYDGKDYIALNEDLRSWTAADTAAQITQRKLEAARAAEQLRAYLEGTCVEWLRRYLENGKETLQRAEPPKTHVTHHPLSDHEATLRCWALGFYPAEITLTWQRDGEDQTQDTELVETRPAGDGTFQKWAAVVVPSGQEQRYTCHMQHEGLQEPLTLSWEPSSQPTIPIMGIVAGLAVLVVLAVLGAVVTAMMCRRKSSGGKGGSCSQAACSNSAQGSDESLITCKA

SEQ ID NO: 68 - protein, 833 aa, Homo sapiens
MYRMQLLSCIALSLALVTNSAPTSSSTKKTQLQLEALLLDLQMILNGINNYKNPKLTRMLTAKFYMPKKATELKHLQCLEEELKPLEEVLNLAQSKNFHLRPRDLISNINVIVLELKGSETTFMCEYADETATIVEFLNRWITFCQSIISTLTGGGGSGGGGSGGGGSGGGGSAPTSSSTKKTQLQLEALLLDLQMILNGINNYKNPKLTRMLTAKFYMPKKATELKHLQCLEEELKPLEEVLNLAQSKNFHLRPRDLISNINVIVLELKGSETTFMCEYADETATIVEFLNRWITFCQSIISTLTGGGGSGGGGSGGGGSGGGGSGSHSMRYFFTSVSRPGRGEPRFIAVGYVDDTQFVRFDSDAASQRMEPRAPWIEQEGPEYWDGETRKVKAHSQTHRVDLGTLRGAYNQSEAGSHTVQRMYGCDVGSDWRFLRGYHQYAYDGKDYIALKEDLRSWTAADMAAQTTKHKWEAAHVAEQLRAYLEGTCVEWLRRYLENGKETLQRTDAPKTHMTHHAVSDHEATLRCWALSFYPAEITLTWQRDGEDQTQDTELVETRPCGDGTFQKWAAVVVPSGQEQRYTCHVQHEGLPKPLTLRWEAAAGGDKTHTCPPCPAPELLGGPSVFLFPPKPKDTLMISRTPEVTCVVVDVSHEDPEVKFNWYVDGVEVHNAKTKPREEQYASTYRVVSVLTVLHQDWLNGKEYKCKVSNKALPAPIEKTISKAKGQPREPQVYTLPPSREEMTKNQVSLTCLVKGFYPSDIAVEWESNGQPENNYKTTPPVLDSDGSFFLYSKLTVDKSRWQQGNVFSCSVMHEALHNHYTQKSLSLSPGK

SEQ ID NO: 69 - protein, 813 aa, Homo sapiens
APTSSSTKKTQLQLEALLLDLQMILNGINNYKNPKLTRMLTAKFYMPKKATELKHLQCLEEELKPLEEVLNLAQSKNFHLRPRDLISNINVIVLELKGSETTFMCEYADETATIVEFLNRWITFCQSIISTLTGGGGSGGGGSGGGGSGGGGSAPTSSSTKKTQLQLEALLLDLQMILNGINNYKNPKLTRMLTAKFYMPKKATELKHLQCLEEELKPLEEVLNLAQSKNFHLRPRDLISNINVIVLELKGSETTFMCEYADETATIVEFLNRWITFCQSIISTLTGGGGSGGGGSGGGGSGGGGSGSHSMRYFFTSVSRPGRGEPRFIAVGYVDDTQFVRFDSDAASQRMEPRAPWIEQEGPEYWDGETRKVKAHSQTHRVDLGTLRGAYNQSEAGSHTVQRMYGCDVGSDWRFLRGYHQYAYDGKDYIALKEDLRSWTAADMAAQTTKHKWEAAHVAEQLRAYLEGTCVEWLRRYLENGKETLQRTDAPKTHMTHHAVSDHEATLRCWALSFYPAEITLTWQRDGEDQTQDTELVETRPCGDGTFQKWAAVVVPSGQEQRYTCHVQHEGLPKPLTLRWEAAAGGDKTHTCPPCPAPELLGGPSVFLFPPKPKDTLMISRTPEVTCVVVDVSHEDPEVKFNWYVDGVEVHNAKTKPREEQYASTYRVVSVLTVLHQDWLNGKEYKCKVSNKALPAPIEKTISKAKGQPREPQVYTLPPSREEMTKNQVSLTCLVKGFYPSDIAVEWESNGQPENNYKTTPPVLDSDGSFFLYSKLTVDKSRWQQGNVFSCSVMHEALHNHYTQKSLSLSPGK

SEQ ID NO: 70 - DNA, 2505 bp, Homo sapiens
atgtacaggatgcaactcctgtcttgcattgcactaagtcttgcacttgtcacaaacagtgcacctacttcaagttctacaaagaaaacacagctacaactggaggcattactgctggatttacagatgattttgaatggaattaataattacaagaatcccaaactcaccaggatgctcacagcaaagttttacatgcccaagaaggccacagaactgaaacatcttcagtgtctagaagaagaactcaaacctctggaggaagtgctaaatttagctcaaagcaaaaactttcacttaagacccagggacttaatcagcaatatcaacgtaatagttctggaactaaagggatctgaaacaacattcatgtgtgaatatgctgatgagacagcaaccattgtagaatttctgaacagatggattaccttttgtcaaagcatcatctcaacactgactggaggcggaggatctggtggtggaggttctggtggtgggggatctggaggcggaggatctgcacctacttcaagttctacaaagaaaacacagctacaactggaggcattactgctggatttacagatgattttgaatggaattaataattacaagaatcccaaactcaccaggatgctcacagcaaagttttacatgcccaagaaggccacagaactgaaacatcttcagtgtctagaagaagaactcaaacctctggaggaagtgctaaatttagctcaaagcaaaaactttcacttaagacccagggacttaatcagcaatatcaacgtaatagttctggaactaaagggatctgaaacaacattcatgtgtgaatatgctgatgagacagcaaccattgtagaatttctgaacagatggattaccttttgtcaaagcatcatctcaacactgactggaggcggaggatctggtggtggaggttctggtggtgggggatctggaggcggaggatctggctctcactccatgaggtatttcttcacatccgtgtcccggcccggccgcggggagccccgcttcatcgcagtgggctacgtggacgacacgcagttcgtgcggttcgacagcgacgccgcgagccagaggatggagccgcgggcgccgtggatagagcaggagggtccggagtattgggacggggagacacggaaagtgaaggcccactcacagactcaccgagtggacctggggaccctgcgcggcgcctacaaccagagcgaggccggttctcacaccgtccagaggatgtatggctgcgacgtggggtcggactggcgcttcctccgcgggtaccaccagtacgcctacgacggcaaggattacatcgccctgaaagaggacctgcgctcttggaccgcggcggacatggcagctcagaccaccaagcacaagtgggaggcggcccatgtggcggagcagttgagagcctacctggagggcacgtgcgtggagtggctccgcagatacctggagaacgggaaggagacgctgcagcgcacggacgcccccaaaacgcatatgactcaccacgctgtctctgaccatgaagccaccctgaggtgctgggccctgagcttctaccctgcggagatcacactgacctggcagcgggatggggaggaccagacccaggacacggagctcgtggagaccaggccttgcggggatggaaccttccagaagtgggcggctgtggtggtgccttctggacaggagcagagatacacctgccatgtgcagcatgagggtttgcccaagcccctcaccctgagatgggaggcagctgcgggtggcgacaaaactcacacatgcccaccgtgcccagcacctgaactcctggggggaccgtcagtcttcctcttccccccaaaacccaaggacaccctcatgatctcccggacccctgaggtcacatgcgtggtggtggacgtgagccacgaagaccctgaggtcaagttcaactggtacgtggacggcgtggaggtgcataatgccaagacaaagccgcgggaggagcagtacgcaagcacgtaccgtgtggtcagcgtcctcaccgtcctgcaccaggactggctgaatggcaaggagtacaagtgcaaggtctccaacaaagccctcccagcccccatcgagaaaaccatctccaaagccaaagggcagccccgagaaccacaggtgtacaccctgcccccatcccgggaggagatgaccaagaaccaggtcagcctgacctgcctggtcaaaggcttctatcccagcgacatcgccgtggagtgggagagcaatgggcagccggagaacaactacaagaccacgcctcccgtgctggactccgacggctccttcttcctctacagcaagctcaccgtggacaagagcagatggcagcaggggaacgtcttctcatgctccgtgatgcacgaggctctgcacaaccactacacgcagaagtccctctccctgtctccgggtaaatagtga

SEQ ID NO: 71 - protein, 833 aa, Homo sapiens
MYRMQLLSCIALSLALVTNSAPTSSSTKKTQLQLEALLLDLQMILNGINNYKNPKLTRMLTAKFYMPKKATELKHLQCLEEELKPLEEVLNLAQSKNFHLRPRDLISNINVIVLELKGSETTFMCEYADETATIVEFLNRWITFCQSIISTLTGGGGSGGGGSGGGGSGGGGSAPTSSSTKKTQLQLEALLLDLQMILNGINNYKNPKLTRMLTAKFYMPKKATELKHLQCLEEELKPLEEVLNLAQSKNFHLRPRDLISNINVIVLELKGSETTFMCEYADETATIVEFLNRWITFCQSIISTLTGGGGSGGGGSGGGGSGGGGSGSHSMRYFFTSVSRPGRGEPRFIAVGYVDDTQFVRFDSDAASQRMEPRAPWIEQEGPEYWDGETRKVKAHSQTHRVDLGTLRGAYNQSEAGSHTVQRMYGCDVGSDWRFLRGYHQYAYDGKDYIALKEDLRSWTAADMAAQTTKHKWEAAHVAEQLRAYLEGTCVEWLRRYLENGKETLQRTDAPKTHMTHHAVSDHEATLRCWALSFYPAEITLTWQRDGEDQTQDTELVETRPCGDGTFQKWAAVVVPSGQEQRYTCHVQHEGLPKPLTLRWEAAAGGDKTHTCPPCPAPEAAGGPSVFLFPPKPKDTLMISRTPEVTCVVVDVSHEDPEVKFNWYVDGVEVHNAKTKPREEQYNSTYRVVSVLTVLHQDWLNGKEYKCKVSNKALPAPIEKTISKAKGQPREPQVYTLPPSREEMTKNQVSLTCLVKGFYPSDIAVEWESNGQPENNYKTTPPVLDSDGSFFLYSKLTVDKSRWQQGNVFSCSVMHEALHNHYTQKSLSLSPGK

SEQ ID NO: 72 - protein, 813 aa, Homo sapiens
APTSSSTKKTQLQLEALLLDLQMILNGINNYKNPKLTRMLTAKFYMPKKATELKHLQCLEEELKPLEEVLNLAQSKNFHLRPRDLISNINVIVLELKGSETTFMCEYADETATIVEFLNRWITFCQSIISTLTGGGGSGGGGSGGGGSGGGGSAPTSSSTKKTQLQLEALLLDLQMILNGINNYKNPKLTRMLTAKFYMPKKATELKHLQCLEEELKPLEEVLNLAQSKNFHLRPRDLISNINVIVLELKGSETTFMCEYADETATIVEFLNRWITFCQSIISTLTGGGGSGGGGSGGGGSGGGGSGSHSMRYFFTSVSRPGRGEPRFIAVGYVDDTQFVRFDSDAASQRMEPRAPWIEQEGPEYWDGETRKVKAHSQTHRVDLGTLRGAYNQSEAGSHTVQRMYGCDVGSDWRFLRGYHQYAYDGKDYIALKEDLRSWTAADMAAQTTKHKWEAAHVAEQLRAYLEGTCVEWLRRYLENGKETLQRTDAPKTHMTHHAVSDHEATLRCWALSFYPAEITLTWQRDGEDQTQDTELVETRPCGDGTFQKWAAVVVPSGQEQRYTCHVQHEGLPKPLTLRWEAAAGGDKTHTCPPCPAPEAAGGPSVFLFPPKPKDTLMISRTPEVTCVVVDVSHEDPEVKFNWYVDGVEVHNAKTKPREEQYNSTYRVVSVLTVLHQDWLNGKEYKCKVSNKALPAPIEKTISKAKGQPREPQVYTLPPSREEMTKNQVSLTCLVKGFYPSDIAVEWESNGQPENNYKTTPPVLDSDGSFFLYSKLTVDKSRWQQGNVFSCSVMHEALHNHYTQKSLSLSPGK

SEQ ID NO: 73 - DNA, 2505 bp, Homo sapiens
atgtacaggatgcaactcctgtcttgcattgcactaagtcttgcacttgtcacaaacagtgcacctacttcaagttctacaaagaaaacacagctacaactggaggcattactgctggatttacagatgattttgaatggaattaataattacaagaatcccaaactcaccaggatgctcacagcaaagttttacatgcccaagaaggccacagaactgaaacatcttcagtgtctagaagaagaactcaaacctctggaggaagtgctaaatttagctcaaagcaaaaactttcacttaagacccagggacttaatcagcaatatcaacgtaatagttctggaactaaagggatctgaaacaacattcatgtgtgaatatgctgatgagacagcaaccattgtagaatttctgaacagatggattaccttttgtcaaagcatcatctcaacactgactggaggcggaggatctggtggtggaggttctggtggtgggggatctggaggcggaggatctgcacctacttcaagttctacaaagaaaacacagctacaactggaggcattactgctggatttacagatgattttgaatggaattaataattacaagaatcccaaactcaccaggatgctcacagcaaagttttacatgcccaagaaggccacagaactgaaacatcttcagtgtctagaagaagaactcaaacctctggaggaagtgctaaatttagctcaaagcaaaaactttcacttaagacccagggacttaatcagcaatatcaacgtaatagttctggaactaaagggatctgaaacaacattcatgtgtgaatatgctgatgagacagcaaccattgtagaatttctgaacagatggattaccttttgtcaaagcatcatctcaacactgactggaggcggaggatctggtggtggaggttctggtggtgggggatctggaggcggaggatctggctctcactccatgaggtatttcttcacatccgtgtcccggcccggccgcggggagccccgcttcatcgcagtgggctacgtggacgacacgcagttcgtgcggttcgacagcgacgccgcgagccagaggatggagccgcgggcgccgtggatagagcaggagggtccggagtattgggacggggagacacggaaagtgaaggcccactcacagactcaccgagtggacctggggaccctgcgcggcgcctacaaccagagcgaggccggttctcacaccgtccagaggatgtatggctgcgacgtggggtcggactggcgcttcctccgcgggtaccaccagtacgcctacgacggcaaggattacatcgccctgaaagaggacctgcgctcttggaccgcggcggacatggcagctcagaccaccaagcacaagtgggaggcggcccatgtggcggagcagttgagagcctacctggagggcacgtgcgtggagtggctccgcagatacctggagaacgggaaggagacgctgcagcgcacggacgcccccaaaacgcatatgactcaccacgctgtctctgaccatgaagccaccctgaggtgctgggccctgagcttctaccctgcggagatcacactgacctggcagcgggatggggaggaccagacccaggacacggagctcgtggagaccaggccttgcggggatggaaccttccagaagtgggcggctgtggtggtgccttctggacaggagcagagatacacctgccatgtgcagcatgagggtttgcccaagcccctcaccctgagatgggaggcagctgcgggtggcgacaaaactcacacatgcccaccgtgcccagcacctgaagccgccgggggaccgtcagtcttcctcttccccccaaaacccaaggacaccctcatgatctcccggacccctgaggtcacatgcgtggtggtggacgtgagccacgaagaccctgaggtcaagttcaactggtacgtggacggcgtggaggtgcataatgccaagacaaagccgcgggaggagcagtacaacagcacgtaccgtgtggtcagcgtcctcaccgtcctgcaccaggactggctgaatggcaaggagtacaagtgcaaggtctccaacaaagccctcccagcccccatcgagaaaaccatctccaaagccaaagggcagccccgagaaccacaggtgtacaccctgcccccatcccgggaggagatgaccaagaaccaggtcagcctgacctgcctggtcaaaggcttctatcccagcgacatcgccgtggagtgggagagcaatgggcagccggagaacaactacaagaccacgcctcccgtgctggactccgacggctccttcttcctctacagcaagctcaccgtggacaagagcagatggcagcaggggaacgtcttctcatgctccgtgatgcacgaggctctgcacaaccactacacgcagaagtccctctccctgtctccgggtaaatagtga

SEQ ID NO: 74 - protein, 833 aa, Homo sapiens
MYRMQLLSCIALSLALVTNSAPTSSSTKKTQLQLEALLLDLQMILNGINNYKNPKLTRMLTAKFYMPKKATELKHLQCLEEELKPLEEVLNLAQSKNFHLRPRDLISNINVIVLELKGSETTFMCEYADETATIVEFLNRWITFCQSIISTLTGGGGSGGGGSGGGGSGGGGSAPTSSSTKKTQLQLEALLLDLQMILNGINNYKNPKLTRMLTAKFYMPKKATELKHLQCLEEELKPLEEVLNLAQSKNFHLRPRDLISNINVIVLELKGSETTFMCEYADETATIVEFLNRWITFCQSIISTLTGGGGSGGGGSGGGGSGGGGSGSHSMRYFFTSVSRPGRGEPRFIAVGYVDDTQFVRFDSDAASQRMEPRAPWIEQEGPEYWDGETRKVKAHSQTHRVDLGTLRGAYNQSEAGSHTVQRMYGCDVGSDWRFLRGYHQYAYDGKDYIALKEDLRSWTAADMAAQTTKHKWEAAHVAEQLRAYLEGTCVEWLRRYLENGKETLQRTDAPKTHMTHHAVSDHEATLRCWALSFYPAEITLTWQRDGEDQTQDTELVETRPCGDGTFQKWAAVVVPSGQEQRYTCHVQHEGLPKPLTLRWEAAAGGDKTHTCPPCPAPEFEGGPSVFLFPPKPKDTLMISRTPEVTCVVVDVSHEDPEVKFNWYVDGVEVHNAKTKPREEQYNSTYRVVSVLTVLHQDWLNGKEYKCKVSNKALPASIEKTISKAKGQPREPQVYTLPPSREEMTKNQVSLTCLVKGFYPSDIAVEWESNGQPENNYKTTPPVLDSDGSFFLYSKLTVDKSRWQQGNVFSCSVMHEALHNHYTQKSLSLSPGK

SEQ ID NO: 75 - protein, 813 aa, Homo sapiens
APTSSSTKKTQLQLEALLLDLQMILNGINNYKNPKLTRMLTAKFYMPKKATELKHLQCLEEELKPLEEVLNLAQSKNFHLRPRDLISNINVIVLELKGSETTFMCEYADETATIVEFLNRWITFCQSIISTLTGGGGSGGGGSGGGGSGGGGSAPTSSSTKKTQLQLEALLLDLQMILNGINNYKNPKLTRMLTAKFYMPKKATELKHLQCLEEELKPLEEVLNLAQSKNFHLRPRDLISNINVIVLELKGSETTFMCEYADETATIVEFLNRWITFCQSIISTLTGGGGSGGGGSGGGGSGGGGSGSHSMRYFFTSVSRPGRGEPRFIAVGYVDDTQFVRFDSDAASQRMEPRAPWIEQEGPEYWDGETRKVKAHSQTHRVDLGTLRGAYNQSEAGSHTVQRMYGCDVGSDWRFLRGYHQYAYDGKDYIALKEDLRSWTAADMAAQTTKHKWEAAHVAEQLRAYLEGTCVEWLRRYLENGKETLQRTDAPKTHMTHHAVSDHEATLRCWALSFYPAEITLTWQRDGEDQTQDTELVETRPCGDGTFQKWAAVVVPSGQEQRYTCHVQHEGLPKPLTLRWEAAAGGDKTHTCPPCPAPEFEGGPSVFLFPPKPKDTLMISRTPEVTCVVVDVSHEDPEVKFNWYVDGVEVHNAKTKPREEQYNSTYRVVSVLTVLHQDWLNGKEYKCKVSNKALPASIEKTISKAKGQPREPQVYTLPPSREEMTKNQVSLTCLVKGFYPSDIAVEWESNGQPENNYKTTPPVLDSDGSFFLYSKLTVDKSRWQQGNVFSCSVMHEALHNHYTQKSLSLSPGK

SEQ ID NO: 76 - DNA, 2505 bp, Homo sapiens
atgtacaggatgcaactcctgtcttgcattgcactaagtcttgcacttgtcacaaacagtgcacctacttcaagttctacaaagaaaacacagctacaactggaggcattactgctggatttacagatgattttgaatggaattaataattacaagaatcccaaactcaccaggatgctcacagcaaagttttacatgcccaagaaggccacagaactgaaacatcttcagtgtctagaagaagaactcaaacctctggaggaagtgctaaatttagctcaaagcaaaaactttcacttaagacccagggacttaatcagcaatatcaacgtaatagttctggaactaaagggatctgaaacaacattcatgtgtgaatatgctgatgagacagcaaccattgtagaatttctgaacagatggattaccttttgtcaaagcatcatctcaacactgactggaggcggaggatctggtggtggaggttctggtggtgggggatctggaggcggaggatctgcacctacttcaagttctacaaagaaaacacagctacaactggaggcattactgctggatttacagatgattttgaatggaattaataattacaagaatcccaaactcaccaggatgctcacagcaaagttttacatgcccaagaaggccacagaactgaaacatcttcagtgtctagaagaagaactcaaacctctggaggaagtgctaaatttagctcaaagcaaaaactttcacttaagacccagggacttaatcagcaatatcaacgtaatagttctggaactaaagggatctgaaacaacattcatgtgtgaatatgctgatgagacagcaaccattgtagaatttctgaacagatggattaccttttgtcaaagcatcatctcaacactgactggaggcggaggatctggtggtggaggttctggtggtgggggatctggaggcggaggatctggctctcactccatgaggtatttcttcacatccgtgtcccggcccggccgcggggagccccgcttcatcgcagtgggctacgtggacgacacgcagttcgtgcggttcgacagcgacgccgcgagccagaggatggagccgcgggcgccgtggatagagcaggagggtccggagtattgggacggggagacacggaaagtgaaggcccactcacagactcaccgagtggacctggggaccctgcgcggcgcctacaaccagagcgaggccggttctcacaccgtccagaggatgtatggctgcgacgtggggtcggactggcgcttcctccgcgggtaccaccagtacgcctacgacggcaaggattacatcgccctgaaagaggacctgcgctcttggaccgcggcggacatggcagctcagaccaccaagcacaagtgggaggcggcccatgtggcggagcagttgagagcctacctggagggcacgtgcgtggagtggctccgcagatacctggagaacgggaaggagacgctgcagcgcacggacgcccccaaaacgcatatgactcaccacgctgtctctgaccatgaagccaccctgaggtgctgggccctgagcttctaccctgcggagatcacactgacctggcagcgggatggggaggaccagacccaggacacggagctcgtggagaccaggccttgcggggatggaaccttccagaagtgggcggctgtggtggtgccttctggacaggagcagagatacacctgccatgtgcagcatgagggtttgcccaagcccctcaccctgagatgggaggcagctgcgggtggcgacaaaactcacacatgcccaccgtgcccagcacctgaattcgaggggggaccgtcagtcttcctcttccccccaaaacccaaggacaccctcatgatctcccggacccctgaggtcacatgcgtggtggtggacgtgagccacgaagaccctgaggtcaagttcaactggtacgtggacggcgtggaggtgcataatgccaagacaaagccgcgggaggagcagtacaacagcacgtaccgtgtggtcagcgtcctcaccgtcctgcaccaggactggctgaatggcaaggagtacaagtgcaaggtctccaacaaagccctcccagccagcatcgagaaaaccatctccaaagccaaagggcagccccgagaaccacaggtgtacaccctgcccccatcccgggaggagatgaccaagaaccaggtcagcctgacctgcctggtcaaaggcttctatcccagcgacatcgccgtggagtgggagagcaatgggcagccggagaacaactacaagaccacgcctcccgtgctggactccgacggctccttcttcctctacagcaagctcaccgtggacaagagcagatggcagcaggggaacgtcttctcatgctccgtgatgcacgaggctctgcacaaccactacacgcagaagtccctctccctgtctccgggtaaatagtga

SEQ ID NO: 77 - protein, 144 aa, Artificial sequence
  Synthetic Polypeptide Sequence
MSRSVALAVLALLSLSGLEAYMLDLQPETTGGGGSGGGGSGGGGSIQRTPKIQVYSCHPAENGKSNFLNCYVSGFHPSDIEVDLLKNGERIEKVEHSDLSFSKDWSFYLLYYTEFTPTEKDEYACRVNHVTLSQPKIVKWDRDM

SEQ ID NO: 78 - protein, 124 aa, Artificial sequence
  Synthetic Polypeptide Sequence
YMLDLQPETTGGGGSGGGGSGGGGSIQRTPKIQVYSCHPAENGKSNFLNCYVSGFHPSDIEVDLLKNGERIEKVEHSDLSFSKDWSFYLLYYTEFTPTEKDEYACRVNHVTLSQPKIVKWDRDM

SEQ ID NO: 79 - DNA, 438 bp, Artificial sequence
  Synthetic Polynucleotide Sequence
atgtctcgctccgtggccttagctgtgctcgcgctactctctctttctggcctggaggcctacatgctcgatttgcagcccgaaacgacgggtggaggtggttctggaggaggcggttcgggcggaggtggtagtatccagcgtactccaaagattcaggtttactcatgccatccagcagagaatggaaagtcaaatttcctgaattgctatgtgtctgggtttcatccatccgacattgaagttgacttactgaagaatggagagagaattgaaaaagtggagcattcagacttgtctttcagcaaggactggtctttctatctcttgtattatactgaattcacccccactgaaaaagatgagtatgcctgccgtgtgaaccacgtgactttgtcacagcccaagatagttaagtgggatcgagacatgtagtga

SEQ ID NO: 80 - protein, 227 aa, Homo sapiens
DKTHTCPPCPAPELLGGPSVFLFPPKPKDTLMISRTPEVTCVVVDVSHEDPEVKFNWYVDGVEVHNAKTKPREEQYNSTYRVVSVLTVLHQDWLNGKEYKCKVSNKALPAPIEKTISKAKGQPREPQVYTLPPSREEMTKNQVSLTCLVKGFYPSDIAVEWESNGQPENNYKTTPPVLDSDGSFFLYSKLTVDKSRWQQGNVFSCSVMHEALHNHYTQKSLSLSPGK

SEQ ID NO: 81 - protein, 227 aa, Homo sapiens
DKTHTCPPCPAPEFEGGPSVFLFPPKPKDTLMISRTPEVTCVVVDVSHEDPEVKFNWYVDGVEVHNAKTKPREEQYNSTYRVVSVLTVLHQDWLNGKEYKCKVSNKALPASIEKTISKAKGQPREPQVYTLPPSREEMTKNQVSLTCLVKGFYPSDIAVEWESNGQPENNYKTTPPVLDSDGSFFLYSKLTVDKSRWQQGNVFSCSVMHEALHNHYTQKSLSLSPGK

SEQ ID NO: 82 - protein, 227 aa, Homo sapiens
DKTHTCPPCPAPELLGGPSVFLFPPKPKDTLMISRTPEVTCVVVDVSHEDPEVKFNWYVDGVEVHNAKTKPREEQYASTYRVVSVLTVLHQDWLNGKEYKCKVSNKALPAPIEKTISKAKGQPREPQVYTLPPSREEMTKNQVSLTCLVKGFYPSDIAVEWESNGQPENNYKTTPPVLDSDGSFFLYSKLTVDKSRWQQGNVFSCSVMHEALHNHYTQKSLSLSPGK

SEQ ID NO: 83 - protein, 227 aa, Homo sapiens
DKTHTCPPCPAPEAAGGPSVFLFPPKPKDTLMISRTPEVTCVVVDVSHEDPEVKFNWYVDGVEVHNAKTKPREEQYNSTYRVVSVLTVLHQDWLNGKEYKCKVSNKALPAPIEKTISKAKGQPREPQVYTLPPSREEMTKNQVSLTCLVKGFYPSDIAVEWESNGQPENNYKTTPPVLDSDGSFFLYSKLTVDKSRWQQGNVFSCSVMHEALHNHYTQKSLSLSPGK

SEQ ID NO: 84 - protein, 133 aa, Homo sapiens
APTSSSTKKTQLQLEALLLDLQMILNGINNYKNPKLTRMLTAKFYMPKKATELKHLQCLEEELKPLEEVLNLAQSKNFHLRPRDLISNINVIVLELKGSETTFMCEYADETATIVEFLNRWITFCQSIISTLT

SEQ ID NO: 85 - protein, 5 aa, Artificial Sequence
  Synthetic Sequence
GSGGS

SEQ ID NO: 86 - protein, 4 aa, Artificial Sequence
  Synthetic Sequence
GGGS

SEQ ID NO: 87 - protein, 9 aa, Artificial Sequence
  Synthetic Peptide
YMLDLQPET

SEQ ID NO: 88 - protein, 4 aa, Artificial Sequence
  Synthetic Sequence
FHHT

SEQ ID NO: 89 - protein, 15 aa, Artificial Sequence
  Synthetic Sequence
GGGGSGGGGSGGGGS

SEQ ID NO: 90 - protein, 20 aa, Artificial Sequence
  Synthetic Sequence
GGGGSGGGGSGGGGSGGGGS

SEQ ID NO: 91 - protein, 25 aa, Artificial Sequence
  Synthetic Sequence
GGGGSGGGGSGGGGSGGGGSGGGGS

SEQ ID NO: 92 - protein, 10 aa, Artificial Sequence
  Synthetic Sequence
GGGGSGGGGS

SEQ ID NO: 93 - protein, 20 aa, Artificial Sequence
  Synthetic Sequence
GSSSSGSSSSGSSSSGSSSS

SEQ ID NO: 94 - protein, 25 aa, Artificial Sequence
  Synthetic Sequence
GSSSSGSSSSGSSSSGSSSSGSSSS

SEQ ID NO: 95 - protein, 119 aa, Homo sapiens
MSRSVALAVLALLSLSGLEAIQRTPKIQVYSRHPAENGKSNFLNCYVSGFHPSDIEVDLLKNGERIEKVEHSDLSFSKDWSFYLLYYTEFTPTEKDEYACRVNHVTLSQPKIVKWDRDM

SEQ ID NO: 96 - protein, 119 aa, Pan troglodytes; identical to SEQ ID NO: 95

SEQ ID NO: 97 - protein, 119 aa, Macaca mulatta
MSRSVALAVLALLSLSGLEAIQRTPKIQVYSRHPPENGKPNFLNCYVSGFHPSDIEVDLLKNGEKMGKVEHSDLSFSKDWSFYLLYYTEFTPNEKDEYACRVNHVTLSGPRTVKWDRDM

SEQ ID NO: 98 - protein, 118 aa, Bos Taurus
MARFVALVLLGLLSLSGLDAIQRPPKIQVYSRHPPEDGKPNYLNCYVYGFHPPQIEIDLLKNGEKIKSEQSDLSFSKDWSFYLLSHAEFTPNSKDQYSCRVKHVTLEQPRIVKWDRDL

SEQ ID NO: 99 - protein, 119 aa, Mus musculus
MARSVTLVFLVLVSLTGLYAIQKTPQIQVYSRHPPENGKPNILNCYVTQFHPPHIEIQMLKNGKKIPKVEMSDMSFSKDWSFYILAHTEFTPTETDTYACRVKHASMAEPKTVYWDRDM

SEQ ID NO: 100 - protein, 5 aa, Artificial Sequence
  Synthetic Sequence
  Misc_Feature (4)..(4): Xaa is an amino acid other than Proline
VPGXG